European Patent Application EP 4 372 089 A1, published May 22, 2024. Title: Chimeric antigen receptor, cell expressing the receptor, pharmaceutical composition containing the cell, method of producing the cell, and polynucleotide or vector containing base sequence encoding the chimeric antigen receptor. Applicant: Noile-Immune Biotech Inc. The sequence listing filed with the application follows.

SEQUENCE LISTING (23 sequences)

SEQ ID NO: 1 - protein, 29 aa, synthetic construct
  REGION 1..29: note = CD8a transmembrane region long
IYIWAPLAGTCGVLLLSLVITLYCNHRNR

SEQ ID NO: 2 - protein, 55 aa, synthetic construct
  REGION 1..55: note = CD8a hinge region long
FVPVFLPAKPTTTPAPRPPTPAPTIASQPLSLRPEACRPAAGGAVHTRGLDFACD

SEQ ID NO: 3 - protein, 19 aa, synthetic construct
  REGION 1..19: note = signal sequence IgG SS long
MDWTWRILFLVAAATGAHS

SEQ ID NO: 4 - protein, 21 aa, synthetic construct
  REGION 1..21: note = signal sequence CD8 SS long
MALPVTALLLPLALLLHAARP

SEQ ID NO: 5 - protein, 45 aa, synthetic construct
  REGION 1..45: note = CD8a hinge region short
TTTPAPRPPTPAPTIASQPLSLRPEACRPAAGGAVHTRGLDFACD

SEQ ID NO: 6 - protein, 253 aa, synthetic construct
  REGION 1..253: note = anti-EGFRviii scFv VL-25-VH humanized
DIVMTQSPLSLPVTPGEPASISCRSSQSLVHSSGKTYLQWYLQKPGQSPQLLIYSVSNRFSGVPDRFSGSGSGRDFTLKISRVEAEDVGVYYCSQSTHVPWTFGGGTKLEIKSSADDAKKDAAKKDDAKKDDAKKDGQVTLKESGPALVKPTQTLTLTCTFSGFSLSTSGMGVSWIRQPPGKALEWLAHIFWDDDKRYNPSLKSRLTISKDTSKNQVVLTMTNMDPVDTATYYCARNYGFDVWGQGTLVTVSS

SEQ ID NO: 7 - protein, 113 aa, Homo sapiens
LRVKFSRSADAPAYQQGQNQLYNELNLGRREEYDVLDKRRGRDPEMGGKPRRKNPQEGLYNELQKDKMAEAYSEIGMKGERRRGKGHDGLYQGLSTATKDTYDALHMQALPPR

SEQ ID NO: 8 - protein, 41 aa, Homo sapiens
RSKRSRLLHSDYMNMTPRRPGPTRKHYQPYAPPRDFAAYRS

SEQ ID NO: 9 - protein, 46 aa, Homo sapiens
RFSVVKRGRKKLLYIFKQPFMRPVQTTQEEDGCSCRFPEEEEGGCE

SEQ ID NO: 10 - protein, 177 aa, Homo sapiens
MFHVSFRYIFGLPPLILVLLPVASSDCDIEGKDGKQYESVLMVSIDQLLDSMKEIGSNCLNNEFNFFKRHICDANKEGMFLFRAARKLRQFLKMNSTGDFDLHLLKVSEGTTILLNCTGQVKGRKPAALGEAQPTKSLEENKSLKEQKKLNDLCFLKRLLQEIKTCWNKILMGTKEH

SEQ ID NO: 11 - protein, 98 aa, Homo sapiens
MALLLALSLLVLWTSPAPTLSGTNDAEDCCLSVTQKPIPGYIVRNFHYLLIKDGCRVPAVVFTTLRGRQLCAPPDQPWVERIIQRLQRTSAKMKRRSS

SEQ ID NO: 12 - protein, 84 aa, Homo sapiens
FVPVFLPAKPTTTPAPRPPTPAPTIASQPLSLRPEACRPAAGGAVHTRGLDFACDIYIWAPLAGTCGVLLLSLVITLYCNHRNR

SEQ ID NO: 13 - protein, 8 aa, synthetic construct
  REGION 1..8: note = 2A peptide cleavage region
  SITE 2: note = misc_feature - Xaa can be any naturally occurring amino acid
  SITE 4: note = misc_feature - Xaa can be any naturally occurring amino acid
DXEXNPGP

SEQ ID NO: 14 - protein, 25 aa, synthetic construct
  REGION 1..25: note = F2A
GSGVKQTLNFDLLKLAGDVESNPGP

SEQ ID NO: 15 - protein, 15 aa, synthetic construct
  REGION 1..15: note = linker 15_aa
GGGGSGGGGSGGGGS

SEQ ID NO: 16 - protein, 25 aa, synthetic construct
  REGION 1..25: note = linker 25_aa
SSADDAKKDAAKKDDAKKDDAKKDG

SEQ ID NO: 17 - DNA, 66 bp, Homo sapiens
  source 1..66: mol_type = genomic DNA
atctacatttgggctcctctggccggaacatgcggagtgctgctgctgagcctcgtgattacactg

SEQ ID NO: 18 - DNA, 339 bp, Homo sapiens
  source 1..339: mol_type = genomic DNA
ctgagagtgaagttcagcaggagcgcagacgcccccgcgtaccagcagggccagaaccagctctataacgagctcaatctaggacgaagagaggagtacgatgttttggacaagagacgtggccgggaccctgagatggggggaaagccgagaaggaagaaccctcaggaaggcctgtacaatgaactgcagaaagataagatggcggaggcctacagtgagattgggatgaaaggcgagcgccggaggggcaaggggcacgatggcctttaccagggtctcagtacagccaccaaggacacctacgacgcccttcacatgcaggccctgccccctcgc

SEQ ID NO: 19 - DNA, 120 bp, Homo sapiens
  source 1..120: mol_type = genomic DNA
agtaagaggagcaggctcctgcacagtgactacatgaacatgactccccgccgccccgggcccacccgcaagcattaccagccctatgccccaccacgcgacttcgcagcctatcgctcc

SEQ ID NO: 20 - DNA, 138 bp, Homo sapiens
  source 1..138: mol_type = genomic DNA
cgtttctctgttgttaaacggggcagaaagaagctcctgtatatattcaaacaaccatttatgagaccagtacaaactactcaagaggaagatggctgtagctgccgatttccagaagaagaagaaggaggatgtgaa

SEQ ID NO: 21 - DNA, 531 bp, Homo sapiens
  source 1..531: mol_type = genomic DNA
atgttccatgtttcttttaggtatatctttggacttcctcccctgatccttgttctgttgccagtagcatcatctgattgtgatattgaaggtaaagatggcaaacaatatgagagtgttctaatggtcagcatcgatcaattattggacagcatgaaagaaattggtagcaattgcctgaataatgaatttaacttttttaaaagacatatctgtgatgctaataaggaaggtatgtttttattccgtgctgctcgcaagttgaggcaatttcttaaaatgaatagcactggtgattttgatctccacttattaaaagtttcagaaggcacaacaatactgttgaactgcactggccaggttaaaggaagaaaaccagctgccctgggtgaagcccaaccaacaaagagtttggaagaaaataaatctttaaaggaacagaaaaaactgaatgacttgtgtttcctaaagagactattacaagagataaaaacttgttggaataaaattttgatgggcactaaagaacac

SEQ ID NO: 22 - DNA, 294 bp, Homo sapiens
  source 1..294: mol_type = genomic DNA
atggccctgctactggccctcagcctgctggttctctggacttccccagccccaactctgagtggcaccaatgatgctgaagactgctgcctgtctgtgacccagaaacccatccctgggtacatcgtgaggaacttccactaccttctcatcaaggatggctgcagggtgcctgctgtagtgttcaccacactgaggggccgccagctctgtgcacccccagaccagccctgggtagaacgcatcatccagagactgcagaggacctcagccaagatgaagcgccgcagcagt

SEQ ID NO: 23 - protein, 67 aa, Homo sapiens
TTTPAPRPPTPAPTIASQPLSLRPEACRPAAGGAVHTRGLDFACDIYIWAPLAGTCGVLLLSLVITL